European Patent Specification EP 4 056 583 B1, published December 11, 2024. Title: Novel Co/Zn/Cd efflux system component variant and a method for producing L-lysine using the same. Applicant: CJ CheilJedang Corporation. The sequence listing filed with the application follows.

SEQUENCE LISTING (10 sequences)

SEQ ID NO: 1 - protein, 205 aa, Artificial Sequence
  (G130D)_Co/Zn/Cd efflux system component
MSEAFDATKVRKAVLTVALLNFAYFFVEFFIALSAGSVSLLADSVDFLEDTSINLLIFIALGWPLARRAVMGKLMAIVILAPAAFAAWAAIQRFSAPQAPEVFPIIVASLGAVVINGASAIIISRVRQHDGSLGQAAFLSARNDVLINIAIIMMALITAWTTSGWPDLILGCFIILLALHAAHEVWEVSEEERLASKALAGEAID

SEQ ID NO: 2 - DNA, 618 bp, Artificial Sequence
  (G130D)_NCgl1992
atgagcgaagcttttgatgcaaccaaagtgcgcaaagctgtgctcaccgtcgcgctgcttaacttcgcttatttctttgtagaattctttattgcattaagcgcaggctccgtttctctactggctgacagtgtcgattttcttgaagacacctccatcaacctgctcattttcattgccctaggatggccgttggcgaggcgcgcagtgatgggcaaacttatggcgattgtgattcttgcacctgctgcttttgctgcgtgggcagcgattcaacggttttccgcaccgcaagcgcccgaagtgtttccgatcatcgtcgcttctctgggcgccgtcgtgatcaacggcgcgagtgccatcattatttctcgagtgcgacaacatgatggctcgcttggccaagctgccttcctatccgcccgaaatgacgtcctgatcaacattgccatcatcatgatggccttaattaccgcatggacgacgtctggatggccagatttgatcctaggttgtttcatcattctgctcgcactgcacgccgctcacgaggtgtgggaagtcagtgaggaagaacgcctcgcctccaaagcccttgctggggaagccatcgattag

SEQ ID NO: 3 - protein, 205 aa, Artificial Sequence
  (WT)_Co/Zn/Cd efflux system component
MSEAFDATKVRKAVLTVALLNFAYFFVEFFIALSAGSVSLLADSVDFLEDTSINLLIFIALGWPLARRAVMGKLMAIVILAPAAFAAWAAIQRFSAPQAPEVFPIIVASLGAVVINGASAIIISRVRQHGGSLGQAAFLSARNDVLINIAIIMMALITAWTTSGWPDLILGCFIILLALHAAHEVWEVSEEERLASKALAGEAID

SEQ ID NO: 4 - DNA, 618 bp, Artificial Sequence
  (WT)_NCgl1992
atgagcgaagcttttgatgcaaccaaagtgcgcaaagctgtgctcaccgtcgcgctgcttaacttcgcttatttctttgtagaattctttattgcattaagcgcaggctccgtttctctactggctgacagtgtcgattttcttgaagacacctccatcaacctgctcattttcattgccctaggatggccgttggcgaggcgcgcagtgatgggcaaacttatggcgattgtgattcttgcacctgctgcttttgctgcgtgggcagcgattcaacggttttccgcaccgcaagcgcccgaagtgtttccgatcatcgtcgcttctctgggcgccgtcgtgatcaacggcgcgagtgccatcattatttctcgagtgcgacaacatggtggctcgcttggccaagctgccttcctatccgcccgaaatgacgtcctgatcaacattgccatcatcatgatggccttaattaccgcatggacgacgtctggatggccagatttgatcctaggttgtttcatcattctgctcgcactgcacgccgctcacgaggtgtgggaagtcagtgaggaagaacgcctcgcctccaaagcccttgctggggaagccatcgattag

SEQ ID NO: 5 - DNA, 40 bp, Artificial Sequence
  NCgl1992_1F
tgaattcgagctcggtaccctttgcgctgtcattgaatgc

SEQ ID NO: 6 - DNA, 33 bp, Artificial Sequence
  NCgl1992_2R
ttggccaagcgagccatcatgttgtcgcactcg

SEQ ID NO: 7 - DNA, 33 bp, Artificial Sequence
  NCgl1992_3F
cgagtgcgacaacatgatggctcgcttggccaa

SEQ ID NO: 8 - DNA, 40 bp, Artificial Sequence
  NCgl1992_4R
gtcgactctagaggatcccccagaggaatcaaacgggcaa

SEQ ID NO: 9 - DNA, 20 bp, Artificial Sequence
  NCgl1992_5F
tttgcgctgtcattgaatgc

SEQ ID NO: 10 - DNA, 19 bp, Artificial Sequence
  NCgl1992_6R
agaggaatcaaacgggcaa